European Patent Application EP 4 335 862 A1, published March 13, 2024. Title: 항암 활성을 가지는 ADP-리보오스 결합 펩티드 및 이의 용도. Applicant: 정근영. The sequence listing filed with the application follows.

SEQUENCE LISTING (28 sequences)

SEQ ID NO: 1 - protein, 25 aa, synthetic construct
  REGION 1..25: note = ADP-ribose binding peptide
VPYIIDLQSMHQFRQDTGTMRPVRR

SEQ ID NO: 2 - protein, 25 aa, synthetic construct
  REGION 1..25: note = ADP-ribose binding peptide
APYIIDLQSMNQFRQDTGTLRPVRR

SEQ ID NO: 3 - protein, 25 aa, synthetic construct
  REGION 1..25: note = ADP-ribose binding peptide
APYIIDLPSWTQFRQDTGTMRAVRR

SEQ ID NO: 4 - protein, 25 aa, synthetic construct
  REGION 1..25: note = ADP-ribose binding peptide
RVYTIDFNSMQQINEDTGTARAIQR

SEQ ID NO: 5 - protein, 25 aa, synthetic construct
  REGION 1..25: note = ADP-ribose binding peptide
FCYLIYFNSMSQMNRQTRRRRRLRR

SEQ ID NO: 6 - protein, 25 aa, synthetic construct
  REGION 1..25: note = ADP-ribose binding peptide
FSYVIDFNTMGQINRQTQRQRRVRR

SEQ ID NO: 7 - protein, 25 aa, synthetic construct
  REGION 1..25: note = ADP-ribose binding peptide
FSYKIDFAEMKQMNLTTGKQRLIKR

SEQ ID NO: 8 - protein, 25 aa, synthetic construct
  REGION 1..25: note = ADP-ribose binding peptide
YNYTVNYTTHTQTNKTSSFCRSVRR

SEQ ID NO: 9 - protein, 24 aa, synthetic construct
  REGION 1..24: note = ADP-ribose binding peptide
RRYTVQFTTMVQVNEETGNRRPVM

SEQ ID NO: 10 - protein, 24 aa, synthetic construct
  REGION 1..24: note = ADP-ribose binding peptide
WIWYWKNESGTWIQYGEEKDKRKN

SEQ ID NO: 11 - protein, 26 aa, synthetic construct
  REGION 1..26: note = ADP-ribose binding peptide
FLYVADLENMVQYRRNEHGRRRKIKR

SEQ ID NO: 12 - protein, 24 aa, synthetic construct
  REGION 1..24: note = ADP-ribose binding peptide
RHYTVNLNTYTATDTKGHSLSVQR

SEQ ID NO: 13 - protein, 26 aa, synthetic construct
  REGION 1..26: note = ADP-ribose binding peptide
GRYDVHLGERMRYAVYWDELASEVRR

SEQ ID NO: 14 - protein, 19 aa, synthetic construct
  REGION 1..19: note = ADP-ribose binding peptide
TAYEASVCDYLEQQVARGN

SEQ ID NO: 15 - protein, 37 aa, synthetic construct
  REGION 1..37: note = ADP-ribose binding peptide with CPP
GRKKRRQRRRPQVPYIIDLQSMHQFRQDTGTMRPVRR

SEQ ID NO: 16 - protein, 37 aa, synthetic construct
  REGION 1..37: note = ADP-ribose binding peptide with CPP
GRKKRRQRRRPQAPYIIDLQSMNQFRQDTGTLRPVRR

SEQ ID NO: 17 - protein, 37 aa, synthetic construct
  REGION 1..37: note = ADP-ribose binding peptide with CPP
GRKKRRQRRRPQAPYIIDLPSWTQFRQDTGTMRAVRR

SEQ ID NO: 18 - protein, 37 aa, synthetic construct
  REGION 1..37: note = ADP-ribose binding peptide with CPP
GRKKRRQRRRPQRVYTIDFNSMQQINEDTGTARAIQR

SEQ ID NO: 19 - protein, 37 aa, synthetic construct
  REGION 1..37: note = ADP-ribose binding peptide with CPP
GRKKRRQRRRPQFCYLIYFNSMSQMNRQTRRRRRLRR

SEQ ID NO: 20 - protein, 37 aa, synthetic construct
  REGION 1..37: note = ADP-ribose binding peptide with CPP
GRKKRRQRRRPQFSYVIDFNTMGQINRQTQRQRRVRR

SEQ ID NO: 21 - protein, 37 aa, synthetic construct
  REGION 1..37: note = ADP-ribose binding peptide with CPP
GRKKRRQRRRPQFSYKIDFAEMKQMNLTTGKQRLIKR

SEQ ID NO: 22 - protein, 37 aa, synthetic construct
  REGION 1..37: note = ADP-ribose binding peptide with CPP
GRKKRRQRRRPQYNYTVNYTTHTQTNKTSSFCRSVRR

SEQ ID NO: 23 - protein, 36 aa, synthetic construct
  REGION 1..36: note = ADP-ribose binding peptide with CPP
GRKKRRQRRRPQRRYTVQFTTMVQVNEETGNRRPVM

SEQ ID NO: 24 - protein, 36 aa, synthetic construct
  REGION 1..36: note = ADP-ribose binding peptide with CPP
GRKKRRQRRRPQWIWYWKNESGTWIQYGEEKDKRKN

SEQ ID NO: 25 - protein, 38 aa, synthetic construct
  REGION 1..38: note = ADP-ribose binding peptide with CPP
GRKKRRQRRRPQFLYVADLENMVQYRRNEHGRRRKIKR

SEQ ID NO: 26 - protein, 36 aa, synthetic construct
  REGION 1..36: note = ADP-ribose binding peptide with CPP
GRKKRRQRRRPQRHYTVNLNTYTATDTKGHSLSVQR

SEQ ID NO: 27 - protein, 38 aa, synthetic construct
  REGION 1..38: note = ADP-ribose binding peptide with CPP
GRKKRRQRRRPQGRYDVHLGERMRYAVYWDELASEVRR

SEQ ID NO: 28 - protein, 31 aa, synthetic construct
  REGION 1..31: note = ADP-ribose binding peptide with CPP
GRKKRRQRRRPQTAYEASVCDYLEQQVARGN